European Patent Application EP 4 112 074 A1, published January 4, 2023. Title: PARENTERAL NOROVIRUS VACCINE FORMULATIONS. Applicant: LigoCyte Pharmaceuticals, Inc. Richardson, Charles Bargatze, Robert F. Mendelman, Paul M. The sequence listing filed with the application follows.

SEQUENCE LISTING (1 sequence)

SEQ ID NO: 1 - protein, 540 aa, Artificial Sequence
  Composite GII.4 Norovirus VP1 amino acid sequence
MKMASSDANPSDGSTANLVPEVNNEVMALEPVVGAAIAAPVAGQQNVIDPWIRNNFVQAPGGEFTVSPRNAPGEILWSAPLGPDLNPYLSHLARMYNGYAGGFEVQVILAGNAFTAGKIIFAAVPPNFPTEGLSPSQVTMFPHIIVDVRQLEPVLIPLPDVRNNFYHYNQSNDPTIKLIAMLYTPLRANNAGDDVFTVSCRVLTRPSPDFDFIFLVPPTVESRTKPFTVPILTVEEMTNSRFPIPLEKLFTGPSGAFVVQPQNGRCTTDGVLLGTTQLSPVNICTFRGDVTHIAGTQEYTMNLASQNWNNYDPTEEIPAPLGTPDFVGKIQGVLTQTTRGDGSTRGHKATVSTGSVHFTPKLGSVQFSTDTSNDFETGQNTKFTPVGVVQDGSTTHQNEPQQWVLPDYSGRDSHNVHLAPAVAPTFPGEQLLFFRSTMPGCSGYPNMNLDCLLPQEWVQHFYQEAAPAQSDVALLRFVNPDTGRVLFECKLHKSGYVTVAHTGQHDLVIPPNGYFRFDSWVNQFYTLAPMGNGTGRRRAL